European Patent Application EP 4 166 563 A1, published April 19, 2023. Title: Bridged nucleoside and nucleotide. Applicant: Liid Pharmaceuticals, Inc. The sequence listing filed with the application follows.

SEQUENCE LISTING (24 sequences)

SEQ ID NO: 1 - DNA, 12 bp, Artificial Sequence
  Single strand
ggatgttctcgt

SEQ ID NO: 2 - DNA, 12 bp, Artificial Sequence
  Oligonucleotide
  misc_difference (6)..(6): Me-TaNA
ggatgttctcgt

SEQ ID NO: 3 - DNA, 12 bp, Artificial Sequence
  Oligonucleotide
  misc_difference (6)..(6): LNA
ggatgttctcgt

SEQ ID NO: 4 - DNA, 12 bp, Artificial Sequence
  Oligonucleotide
  misc_difference (6)..(6): ENA
ggatgttctcgt

SEQ ID NO: 5 - DNA, 12 bp, Artificial Sequence
  Oligonucleotide
  misc_difference (6)..(6): Me-TaNA
  misc_difference (7)..(7): Me-TaNA
ggatgttctcgt

SEQ ID NO: 6 - DNA, 12 bp, Artificial Sequence
  Oligonucleotide
  misc_difference (6)..(6): LNA
  misc_difference (7)..(7): LNA
ggatgttctcgt

SEQ ID NO: 7 - DNA, 12 bp, Artificial Sequence
  Oligonucleotide
  misc_difference (6)..(6): ENA
  misc_difference (7)..(7): ENA
ggatgttctcgt

SEQ ID NO: 8 - DNA, 12 bp, Artificial Sequence
  Oligonucleotide
  misc_difference (4)..(4): Me-TaNA
  misc_difference (6)..(6): Me-TaNA
ggatgttctcgt

SEQ ID NO: 9 - DNA, 12 bp, Artificial Sequence
  Oligonucleotide
  misc_difference (4)..(4): LNA
  misc_difference (6)..(6): LNA
ggatgttctcgt

SEQ ID NO: 10 - DNA, 12 bp, Artificial Sequence
  Oligonucleotide
  misc_difference (4)..(4): ENA
  misc_difference (6)..(6): ENA
ggatgttctcgt

SEQ ID NO: 11 - RNA, 12 nt, Artificial Sequence
  RNA
acgagaacaucc

SEQ ID NO: 12 - DNA, 12 bp, Artificial Sequence
  DNA
acgagaacatcc

SEQ ID NO: 13 - DNA, 14 bp, Artificial Sequence
  Single strand
  misc_feature (2)..(2): 2'-Deoxy-5-methylcytidine
  misc_feature (5)..(5): 2'-Deoxy-5-methylcytidine
  misc_feature (11)..(11): 2'-Deoxy-5-methylcytidine
  misc_feature (13)..(13): 2'-Deoxy-5-methylcytidine
tcttctttttctct

SEQ ID NO: 14 - DNA, 14 bp, Artificial Sequence
  Oligonucleotide
  misc_feature (2)..(2): 2'-Deoxy-5-methylcytidine
  misc_feature (5)..(5): 2'-Deoxy-5-methylcytidine
  misc_difference (8)..(8): Me-TaNA
  misc_feature (11)..(11): 2'-Deoxy-5-methylcytidine
  misc_feature (13)..(13): 2'-Deoxy-5-methylcytidine
tcttctttttctct

SEQ ID NO: 15 - DNA, 14 bp, Artificial Sequence
  Oligonucleotide
  misc_feature (2)..(2): 2'-Deoxy-5-methylcytidine
  misc_feature (5)..(5): 2'-Deoxy-5-methylcytidine
  misc_difference (8)..(8): LNA
  misc_feature (11)..(11): 2'-Deoxy-5-methylcytidine
  misc_feature (13)..(13): 2'-Deoxy-5-methylcytidine
tcttctttttctct

SEQ ID NO: 16 - DNA, 14 bp, Artificial Sequence
  Oligonucleotide
  misc_feature (2)..(2): 2'-Deoxy-5-methylcytidine
  misc_feature (5)..(5): 2'-Deoxy-5-methylcytidine
  misc_difference (8)..(8): ENA
  misc_feature (11)..(11): 2'-Deoxy-5-methylcytidine
  misc_feature (13)..(13): 2'-Deoxy-5-methylcytidine
tcttctttttctct

SEQ ID NO: 17 - DNA, 14 bp, Artificial Sequence
  Oligonucleotide
  misc_feature (2)..(2): 2'-Deoxy-5-methylcytidine
  misc_feature (5)..(5): 2'-Deoxy-5-methylcytidine
  misc_difference (7)..(7): Me-TaNA
  misc_difference (8)..(8): Me-TaNA
  misc_difference (9)..(9): Me-TaNA
  misc_feature (11)..(11): 2'-Deoxy-5-methylcytidine
  misc_feature (13)..(13): 2'-Deoxy-5-methylcytidine
tcttctttttctct

SEQ ID NO: 18 - DNA, 14 bp, Artificial Sequence
  Oligonucleotide
  misc_feature (2)..(2): 2'-Deoxy-5-methylcytidine
  misc_feature (5)..(5): 2'-Deoxy-5-methylcytidine
  misc_difference (7)..(7): LNA
  misc_difference (8)..(8): LNA
  misc_difference (9)..(9): LNA
  misc_feature (11)..(11): 2'-Deoxy-5-methylcytidine
  misc_feature (13)..(13): 2'-Deoxy-5-methylcytidine
tcttctttttctct

SEQ ID NO: 19 - DNA, 14 bp, Artificial Sequence
  Oligonucleotide
  misc_feature (2)..(2): 2'-Deoxy-5-methylcytidine
  misc_feature (5)..(5): 2'-Deoxy-5-methylcytidine
  misc_difference (7)..(7): ENA
  misc_difference (8)..(8): ENA
  misc_difference (9)..(9): ENA
  misc_feature (11)..(11): 2'-Deoxy-5-methylcytidine
  misc_feature (13)..(13): 2'-Deoxy-5-methylcytidine
tcttctttttctct

SEQ ID NO: 20 - DNA, 14 bp, Artificial Sequence
  Oligonucleotide
  misc_feature (2)..(2): 2'-Deoxy-5-methylcytidine
  misc_feature (5)..(5): 2'-Deoxy-5-methylcytidine
  misc_difference (6)..(6): Me-TaNA
  misc_difference (8)..(8): Me-TaNA
  misc_difference (10)..(10): Me-TaNA
  misc_feature (11)..(11): 2'-Deoxy-5-methylcytidine
  misc_feature (13)..(13): 2'-Deoxy-5-methylcytidine
tcttctttttctct

SEQ ID NO: 21 - DNA, 14 bp, Artificial Sequence
  Oligonucleotide
  misc_feature (2)..(2): 2'-Deoxy-5-methylcytidine
  misc_feature (5)..(5): 2'-Deoxy-5-methylcytidine
  misc_difference (6)..(6): LNA
  misc_difference (8)..(8): LNA
  misc_difference (10)..(10): LNA
  misc_feature (11)..(11): 2'-Deoxy-5-methylcytidine
  misc_feature (13)..(13): 2'-Deoxy-5-methylcytidine
tcttctttttctct

SEQ ID NO: 22 - DNA, 14 bp, Artificial Sequence
  Oligonucleotide
  misc_feature (2)..(2): 2'-Deoxy-5-methylcytidine
  misc_feature (5)..(5): 2'-Deoxy-5-methylcytidine
  misc_difference (6)..(6): ENA
  misc_difference (8)..(8): ENA
  misc_difference (10)..(10): ENA
  misc_feature (11)..(11): 2'-Deoxy-5-methylcytidine
  misc_feature (13)..(13): 2'-Deoxy-5-methylcytidine
tcttctttttctct

SEQ ID NO: 23 - DNA, 40 bp, Artificial Sequence
  Strand of hairpin double-stranded DNA
  misc_structure (20)..(21): C18spacer
ggcagaagaaaaagagacgcgcgtctctttttcttctgcc

SEQ ID NO: 24 - DNA, 10 bp, Artificial Sequence
  Test Oligonucleotide
tttttttttt